European Patent Specification EP 3 371 307 B1, published December 4, 2024. Title: PAENIBACILLUS AND BACILLUS SPP. MANNANASES. Applicant: Danisco US, Inc. The sequence listing filed with the application follows.

SEQUENCE LISTING (29 sequences)

SEQ ID NO: 1 - DNA, 894 bp, artificial sequence
  synthetic
atggcgacaggcttttatgtttcaggcaacaaactgtatgatagcacaggcaaaccgtttgttatgagaggcgttaatcatggccatagctggtttaaaaacgatctgaatacagcgattccggctattgcaaaaacaggcgcaaatacagttagaattgttctgtcaaatggcagcctgtatacgaaagatgatctgaatgcagtcaaaaacatcatcaatgtcgtcaaccagaacaaaatgattgcagttctggaagttcatgatgcaacgggcaaagatgattacaattcactggatgcagcagtcaactattggatctcaattaaagaagcgctgatcggcaaagaagatcgcgttattgttaatattgcgaacgaatggtatggcacatggaatggctcagcatgggcagatggctacaaaaaagcaattccgaaactgagaaatgcaggcatcaaaaacacactgattgttgatgcggcaggctggggacaatttccgcaatcaattgttgattatggccaaagcgtttttgcagcagatagccagaaaaatacagtctttagcatccatatgtacgaatacgctggaaaagatgcagcaacagttaaagcgaatatggaaaacgtcctgaataaaggcctggcactgattattggcgaatttggcggatatcatacaaatggcgacgttgatgaatatgcgattatgagatatggccaagaaaaaggcgttggctggcttgcatggtcatggtatggaaattcatcaggccttaactatctggatatggcaacaggaccgaatggatcactgacatcatttggcaatacagtcgtcaatgatacgtatggaatcaaaaatacgagccagaaagctggcatcttttaa

SEQ ID NO: 2 - protein, 297 aa, artificial sequence
  synthetic
MATGFYVSGNKLYDSTGKPFVMRGVNHGHSWFKNDLNTAIPAIAKTGANTVRIVLSNGSLYTKDDLNAVKNIINVVNQNKMIAVLEVHDATGKDDYNSLDAAVNYWISIKEALIGKEDRVIVNIANEWYGTWNGSAWADGYKKAIPKLRNAGIKNTLIVDAAGWGQFPQSIVDYGQSVFAADSQKNTVFSIHMYEYAGKDAATVKANMENVLNKGLALIIGEFGGYHTNGDVDEYAIMRYGQEKGVGWLAWSWYGNSSGLNYLDMATGPNGSLTSFGNTVVNDTYGIKNTSQKAGIF

SEQ ID NO: 3 - DNA, 608 bp, Bacillus subtilis
gaattctccattttcttctgctatcaaaataacagactcgtgattttccaaacgagctttcaaaaaagcctctgccccttgcaaatcggatgcctgtctataaaattcccgatattggttaaacagcggcgcaatggcggccgcatctgatgtctttgcttggcgaatgttcatcttatttcttcctccctctcaataattttttcattctatcccttttctgtaaagtttatttttcagaatacttttatcatcatgctttgaaaaaatatcacgataatatccattgttctcacggaagcacacgcaggtcatttgaacgaattttttcgacaggaatttgccgggactcaggagcatttaacctaaaaaagcatgacatttcagcataatgaacatttactcatgtctattttcgttcttttctgtatgaaaatagttatttcgagtctctacggaaatagcgagagatgatatacctaaatagagataaaatcatctcaaaaaaatgggtctactaaaatattattccatctattacaataaattcacagaatagtcttttaagtaagtctactctgaatttttttaaaaggagagggtaaaga

SEQ ID NO: 4 - DNA, 87 bp, Bacillus subtilis
gtgagaagcaaaaaattgtggatcagcttgttgtttgcgttaacgttaatctttacgatggcgttcagcaacatgtctgctagcgca

SEQ ID NO: 5 - DNA, 93 bp, artificial sequence
  terminator
ggttaccttgaatgtatataaacattctcaaagggatttctaataaaaaacgctcggttgccgccgggcgttttttatgcatcgatggaattc

SEQ ID NO: 6 - protein, 297 aa, artificial sequence
  variant
MATGFYVSGNKLYDSTGKEFVMRGVNHGHSWFKNDLNEAIPAIAKTGANTVRIVLSNGSLYTKDDLDAVKNIINVVNQNKMIAVLEVHDATGKDDYDSLDAAVNYWISIKEALIGKEDRVIVNIANEWMGTWNGSAWADGYKKAIPKLRNAGIKNTLIVDAAGWGQFSQSIVDYGQSVFAADSLKNTVFSIHMYEYAGKDAATVKANMENVLNKGLALIIGEFGGYHTNGDVDEYAIMRYGQELGVGWLAWSWYGNSDGLRYLDMATGPNGSLTSFGNTVVNDTYGIKNTSQKAGIF

SEQ ID NO: 7 - protein, 298 aa, artificial sequence
  variant
MATGFYVSGTKLYDSTGKEFVMRGVNHGHTWFKNDLNEAIPAIAKTGANTVRIVLSNGVQYTRDDLDAVKNIINVVNQNKMIAVLEVHDATGKDDYDSLDAAVNYWISIKEALIGKEDRVIVNIANEWMGTWNGSAWADGYKQAIPKLRNAGIKNTLIVDAAGWGQFSQSIVDYGQSVFAADSLKNTVFSIHMYEYAGKDAATVKANMENVLNKGLALIIGEFGPYHVNGDVDELAIMRYGQELGVGWLAWSWYGNSDGLRYLDMATGPNGSLTSFGNTVVNDTYGIKNTSQKAGIFQ

SEQ ID NO: 8 - protein, 309 aa, unknown
  Bacillus sp.
ANSGFYVSGTTLYDANGNPFVMRGINHGHAWYKDQATTAIEGIANTGANTVRIVLSDGGQWTKDDIHTVRNLISLAEDNHLVAVLEVHDATGYDSIASLNRAVDYWIEMRSALIGKEDTVIINIANEWFGSWEGDAWADGYKQAIPRLRNAGLNHTLMVDAAGWGQFPQSIHDYGREVFNADPQRNTMFSIHMYEYAGGNASQVRTNIDRVLNQDLALVIGEFGHRHTNGDVDEATIMSYSEQRGVGWLAWSWKGNGPEWEYLDLSNDWAGNNLTAWGNTIVNGPYGLRETSRLSTVFTGGGSDGGTSP

SEQ ID NO: 9 - protein, 293 aa, Bacillus agaradhaerens
GFSVDGNTLYDANGQPFVMRGINHGHAWYKDTASTAIPAIAEQGANTIRIVLSDGGQWEKDDIDTIREVIELAEQNKMVAVVEVHDATGRDSRSDLNRAVDYWIEMKDALIGKEDTVIINIANEWYGSWDGSAWADGYIDVIPKLRDAGLTHTLMVDAAGWGQYPQSIHDYGQDVFNADPLKNTMFSIHMYEYAGGDANTVRSNIDRVIDQDLALVIGEFGHRHTDVDEDTILSYSEETGTGWLAWSWKGNSTSWDYLDLSEDWAGQHLTDWGNRIVHGADGLQETSKPSTVF

SEQ ID NO: 10 - protein, 299 aa, unknown
  Bacillus sp. JAMB-602
NSGFYVSGTTLYDANGNPFVMRGINHGHAWYKDQATTAIEGIANTGANTVRIVLSDGGQWTKDDIQTVRNLISLAEDNNLVAVLEVHDATGYDSIASLNRAVDYWIEMRSALIGKEDTVIINIANEWFGSWDGAAWADGYKQAIPRLRNAGLNNTLMIDAAGWGQFPQSIHDYGREVFNADPQRNTMFSIHMYEYAGGNASQVRTNIDRVLNQDLALVIGEFGHRHTNGDVDESTIMSYSEQRGVGWLAWSWKGNGPEWEYLDLSNDWAGNNLTAWGNTIVNGPYGLRETSKLSTVFTG

SEQ ID NO: 11 - protein, 10 aa, artificial sequence
  Motif
  MISC_FEATURE (2)..(2): X is F or Y
  MISC_FEATURE (7)..(8): X is any amino acid
WXKNDLXXAI

SEQ ID NO: 12 - protein, 12 aa, artificial sequence
  motif
  MISC_FEATURE (3)..(5): X is any amino acid
  MISC_FEATURE (8)..(8): X is any amino acid
  MISC_FEATURE (10)..(10): X is any amino acid
LDXXXGPXGXLT

SEQ ID NO: 13 - protein, 12 aa, artificial sequence
  motif
  MISC_FEATURE (3)..(3): X is M or L
  MISC_FEATURE (4)..(4): X is V or A
  MISC_FEATURE (5)..(5): X is T or A
  MISC_FEATURE (8)..(8): X is N, A or S
  MISC_FEATURE (10)..(10): X is N, S or T
LDXXXGPXGXLT

SEQ ID NO: 14 - protein, 12 aa, artificial sequence
  motif
  MISC_FEATURE (3)..(3): X is M or L
  MISC_FEATURE (8)..(8): X is N or A
  MISC_FEATURE (10)..(10): X is S or T
LDXATGPXGXLT

SEQ ID NO: 15 - protein, 299 aa, unknown
  Bacillus sp.
ANSGFYVSGTTLYDANGNPFVMRGINHGHAWYKDQATTAIEGIANTGANTVRIVLSDGGQWTKDDIHTVRNLISLAEDNHLVAVPEVHDATGYDSIASLNRAVDYWIEMRSALIGKEDTVIINIANEWFGSWEGDAWADGYKQAIPRLRNAGLNHTLMVDAAGWGQFPQSIHDYGREVFNADPQRNTMFSIHMYEYAGGNASQVRTNIDRVLNQDLALVIGEFGHRHTNGDVDEATIMSYSEQRGVGWLAWSWKGNGPEWEYLDLSNDWAGNNLTAWGNTIVNGPYGLRETSRLSTVFT

SEQ ID NO: 16 - protein, 312 aa, artificial sequence
  synthetic
AGKANSGFYVSGTTLYDANGNPFVMRGINHGHAWYKDQATTAIEGIANTGANTVRIVLSDGGQWTKDDIHTVRNLISLAEDNHLVAVLEVHDATGYDSIASLNRAVDYWIEMRSALIGKEDTVIINIANEWFGSWEGDAWADGYKQAIPRLRNAGLNHTLMVDAAGWGQFPQSIHDYGREVFNADPQRNTMFSIHMYEYAGGNASQVRTNIDRVLNQDLALVIGEFGHRHTNGDVDEATIMSYSEQRGVGWLAWSWKGNGPEWEYLDLSNDWAGNNLTAWGNTIVNGPYGLRETSRLSTVFTGGGSDGGTSP

SEQ ID NO: 17 - protein, 309 aa, unknown
  Bacillus sp.
ANSGFYVSGTTLYDANGNPFVMRGINHGHAWYKDQATTAIEGIANTGANTVRIVLSDGGQWTKDDIHTVRNLISLAEDNHLVAVPEVHDATGYDSIASLNRAVDYWIEMRSALIGKEDTVIINIANEWFGSWEGDAWADGYKQAIPRLRNAGLNHTLMVDAAGWGQFPQSIHDYGREVFNADPQRNTMFSIHMYEYAGGNASQVRTNIDRVLNQDLALVIGEFGHRHTNGDVDEATIMSYSEQRGVGWLAWSWKGNGPEWEYLDLSNDWAGNNLTAWGNTIVNGPYGLRETSRLSTVFTGGGSDGGTSP

SEQ ID NO: 18 - DNA, 1023 bp, artificial sequence
  synthetic
gtgagaagcaaaaaattgtggatcagcttgttgtttgcgttaacgttaatctttacgatggcgttcagcaacatgagcgcgcaggctgctggaaaagcaaactcaggcttttatgtttcaggcacaacactgtacgacgcaaatggcaatccgtttgttatgagaggcattaaccatggacatgcctggtataaagatcaagcaacaacagcgattgaaggcattgcaaatacaggcgcaaacacagtgagaattgttctttcagacggaggccaatggacaaaagatgatattcatacggttagaaatctgatttcactggcagaggataatcatctggttgcagttctggaagttcatgatgcaacaggctatgattcaattgcaagccttaatagagcagttgattattggattgaaatgagatcagcactgattggcaaagaagatacagtcatcattaacattgccaacgaatggtttggctcatgggaaggcgatgcatgggcagacggctataagcaagcaattccgagactgagaaatgcaggacttaatcatacactgatggttgatgcagcaggctggggccagttcccgcaatcaattcacgattatggaagagaggtttttaacgcagatccgcagagaaatacaatgtttagcattcatatgtacgaatatgcaggcggcaacgcatcacaagttagaacaaatattgatagagttctgaaccaggatctggcactggttatcggagaatttggccatagacatacgaacggcgatgttgatgaagctacaattatgtcatactcagaacagagaggcgtcggatggctggcatggtcatggaaaggcaacggaccggaatgggaatatctggatctgtcaaatgattgggcaggaaataacctgacagcatggggcaatacgattgttaacggcccgtatggcctgagagaaacatcaagactgtcaacagtttttacaggaggcggatcagatggcggcacatcaccg

SEQ ID NO: 19 - protein, 341 aa, artificial sequence
  synthetic
MRSKKLWISLLFALTLIFTMAFSNMSAQAAGKANSGFYVSGTTLYDANGNPFVMRGINHGHAWYKDQATTAIEGIANTGANTVRIVLSDGGQWTKDDIHTVRNLISLAEDNHLVAVLEVHDATGYDSIASLNRAVDYWIEMRSALIGKEDTVIINIANEWFGSWEGDAWADGYKQAIPRLRNAGLNHTLMVDAAGWGQFPQSIHDYGREVFNADPQRNTMFSIHMYEYAGGNASQVRTNIDRVLNQDLALVIGEFGHRHTNGDVDEATIMSYSEQRGVGWLAWSWKGNGPEWEYLDLSNDWAGNNLTAWGNTIVNGPYGLRETSRLSTVFTGGGSDGGTSP

SEQ ID NO: 20 - protein, 312 aa, artificial sequence
  BspMan5 variant
AGKANSGFYVSGTTLYDANGNEFVMRGINHGHAWYKDQATTAIEGIANTGANTVRIVLSDGGQWTKDDIHTVRNLISLAEDNHLVAVLEVHDATGYDSIASLNRAVDYWIEMRSALIGKEDTVIINIANEWFGSWEGDAWADGYKQAIPRLRNAGLNHTLMVDAAGWGQFPQSIHDYGREVFNADPQRNTMFSIHMYEYAGGNASQVRTNIDRVLNQDLALVIGEFGHRHTNGDVDEATIMSYSEQRGVGWLAWSWKGNGPEWEYLDLSNDWAGNNLTAWGNTIVNGPYGLRETSRLSTVFTGGGSDGGTSP

SEQ ID NO: 21 - protein, 312 aa, artificial sequence
  BspMan5 variant
AGKANSGFYVSGTTLYDANGNPFVMRGINHGHAWYKDQATEAIEGIANTGANTVRIVLSDGGQWTKDDIHTVRNLISLAEDNHLVAVLEVHDATGYDSIASLNRAVDYWIEMRSALIGKEDTVIINIANEWFGSWEGDAWADGYKQAIPRLRNAGLNHTLMVDAAGWGQFPQSIHDYGREVFNADPQRNTMFSIHMYEYAGGNASQVRTNIDRVLNQDLALVIGEFGHRHTNGDVDEATIMSYSEQRGVGWLAWSWKGNGPEWEYLDLSNDWAGNNLTAWGNTIVNGPYGLRETSRLSTVFTGGGSDGGTSP

SEQ ID NO: 22 - protein, 312 aa, artificial sequence
  BspMan5 variant
AGKANSGFYVSGTTLYDANGNPFVMRGINHGHAWYKDQATTAIEGIANTGANTVRIVLSDGGQWTKDDIDTVRNLISLAEDNHLVAVLEVHDATGYDSIASLNRAVDYWIEMRSALIGKEDTVIINIANEWFGSWEGDAWADGYKQAIPRLRNAGLNHTLMVDAAGWGQFPQSIHDYGREVFNADPQRNTMFSIHMYEYAGGNASQVRTNIDRVLNQDLALVIGEFGHRHTNGDVDEATIMSYSEQRGVGWLAWSWKGNGPEWEYLDLSNDWAGNNLTAWGNTIVNGPYGLRETSRLSTVFTGGGSDGGTSP

SEQ ID NO: 23 - protein, 312 aa, artificial sequence
  BspMan5 variant
AGKANSGFYVSGTTLYDANGNPFVMRGINHGHAWYKDQATTAIEGIANTGANTVRIVLSDGGQWTKDDIHTVRNLISLAEDNHLVAVLEVHDATGYDSIASLNRAVDYWIEMRSALIGKEDTVIINIANEWMGSWEGDAWADGYKQAIPRLRNAGLNHTLMVDAAGWGQFPQSIHDYGREVFNADPQRNTMFSIHMYEYAGGNASQVRTNIDRVLNQDLALVIGEFGHRHTNGDVDEATIMSYSEQRGVGWLAWSWKGNGPEWEYLDLSNDWAGNNLTAWGNTIVNGPYGLRETSRLSTVFTGGGSDGGTSP

SEQ ID NO: 24 - protein, 312 aa, artificial sequence
  BspMan5 variant
AGKANSGFYVSGTTLYDANGNPFVMRGINHGHAWYKDQATTAIEGIANTGANTVRIVLSDGGQWTKDDIHTVRNLISLAEDNHLVAVLEVHDATGYDSIASLNRAVDYWIEMRSALIGKEDTVIINIANEWFGSWEGDAWADGYKQAIPRLRNAGLNHTLMVDAAGWGQFSQSIHDYGREVFNADPQRNTMFSIHMYEYAGGNASQVRTNIDRVLNQDLALVIGEFGHRHTNGDVDEATIMSYSEQRGVGWLAWSWKGNGPEWEYLDLSNDWAGNNLTAWGNTIVNGPYGLRETSRLSTVFTGGGSDGGTSP

SEQ ID NO: 25 - protein, 312 aa, artificial sequence
  BspMan5 variant
AGKANSGFYVSGTTLYDANGNPFVMRGINHGHAWYKDQATTAIEGIANTGANTVRIVLSDGGQWTKDDIHTVRNLISLAEDNHLVAVLEVHDATGYDSIASLNRAVDYWIEMRSALIGKEDTVIINIANEWFGSWEGDAWADGYKQAIPRLRNAGLNHTLMVDAAGWGQFPQSIHDYGREVFNADPLRNTMFSIHMYEYAGGNASQVRTNIDRVLNQDLALVIGEFGHRHTNGDVDEATIMSYSEQRGVGWLAWSWKGNGPEWEYLDLSNDWAGNNLTAWGNTIVNGPYGLRETSRLSTVFTGGGSDGGTSP

SEQ ID NO: 26 - protein, 312 aa, artificial sequence
  BspMan5 variant
AGKANSGFYVSGTTLYDANGNPFVMRGINHGHAWYKDQATTAIEGIANTGANTVRIVLSDGGQWTKDDIHTVRNLISLAEDNHLVAVLEVHDATGYDSIASLNRAVDYWIEMRSALIGKEDTVIINIANEWFGSWEGDAWADGYKQAIPRLRNAGLNHTLMVDAAGWGQFPQSIHDYGREVFNADPQRNTMFSIHMYEYAGGNASQVRTNIDRVLNQDLALVIGEFGPRHTNGDVDEATIMSYSEQRGVGWLAWSWKGNGPEWEYLDLSNDWAGNNLTAWGNTIVNGPYGLRETSRLSTVFTGGGSDGGTSP

SEQ ID NO: 27 - protein, 312 aa, artificial sequence
  BspMan5 variant
AGKANSGFYVSGTTLYDANGNPFVMRGINHGHAWYKDQATTAIEGIANTGANTVRIVLSDGGQWTKDDIHTVRNLISLAEDNHLVAVLEVHDATGYDSIASLNRAVDYWIEMRSALIGKEDTVIINIANEWFGSWEGDAWADGYKQAIPRLRNAGLNHTLMVDAAGWGQFPQSIHDYGREVFNADPQRNTMFSIHMYEYAGGNASQVRTNIDRVLNQDLALVIGEFGHRHTNGDVDEATIMSYSEQLGVGWLAWSWKGNGPEWEYLDLSNDWAGNNLTAWGNTIVNGPYGLRETSRLSTVFTGGGSDGGTSP

SEQ ID NO: 28 - protein, 312 aa, artificial sequence
  BspMan5 variant
AGKANSGFYVSGTTLYDANGNPFVMRGINHGHAWYKDQATTAIEGIANTGANTVRIVLSDGGQWTKDDIHTVRNLISLAEDNHLVAVLEVHDATGYDSIASLNRAVDYWIEMRSALIGKEDTVIINIANEWFGSWEGDAWADGYKQAIPRLRNAGLNHTLMVDAAGWGQFPQSIHDYGREVFNADPQRNTMFSIHMYEYAGGNASQVRTNIDRVLNQDLALVIGEFGHRHTNGDVDEATIMSYSEQRGVGWLAWSWKGNGDEWEYLDLSNDWAGNNLTAWGNTIVNGPYGLRETSRLSTVFTGGGSDGGTSP

SEQ ID NO: 29 - protein, 312 aa, artificial sequence
  BspMan5 variant
AGKANSGFYVSGTTLYDANGNPFVMRGINHGHAWYKDQATTAIEGIANTGANTVRIVLSDGGQWTKDDIHTVRNLISLAEDNHLVAVLEVHDATGYDSIASLNRAVDYWIEMRSALIGKEDTVIINIANEWFGSWEGDAWADGYKQAIPRLRNAGLNHTLMVDAAGWGQFPQSIHDYGREVFNADPQRNTMFSIHMYEYAGGNASQVRTNIDRVLNQDLALVIGEFGHRHTNGDVDEATIMSYSEQRGVGWLAWSWKGNGPEWRYLDLSNDWAGNNLTAWGNTIVNGPYGLRETSRLSTVFTGGGSDGGTSP